European Patent Application EP 4 238 980 A1, published September 6, 2023. Title: PEPTIDES WITH PLANT PROTECTION ACTION. Applicant: Università degli studi di Padova. The sequence listing filed with the application follows.

SEQUENCE LISTING (16 sequences)

SEQ ID NO: 1 - protein, 11 aa, synthetic construct
  SITE 1: note = 1 ottanoile Aib
  REGION 1..11: note = Designed peptide K259G6
  SITE 2: note = Lys(HCl)
  SITE 4: note = Aib
  SITE 5: note = Lys(HCl)
  SITE 8: note = Aib
  SITE 9: note = Lys(HCl)
  SITE 11: note = Lol
XXLXXGLXXIX

SEQ ID NO: 2 - protein, 11 aa, synthetic construct
  SITE 1: note = 1 ottanoile Aib
  REGION 1..11: note = Designed peptide K259G6-NH2
  SITE 2: note = Lys(HCl)
  SITE 4: note = Aib
  SITE 5: note = Lys(HCl)
  SITE 8: note = Aib
  SITE 9: note = Lys(HCl)
XXLXXGLXXIL

SEQ ID NO: 3 - skipped

SEQ ID NO: 4 - protein, 11 aa, synthetic construct
  SITE 1: note = 1 ottanoile Aib
  REGION 1..11: note = Designed peptide K2569-NH2
  SITE 2: note = Lys(HCl)
  SITE 4: note = Aib
  SITE 5: note = Lys(HCl)
  SITE 6: note = Lys(HCl)
  SITE 8: note = Aib
  SITE 9: note = Lys(HCl)
XXLXXXLXXIL

SEQ ID NO: 5 - protein, 11 aa, synthetic construct
  SITE 1: note = 1 ottanoile Aib
  REGION 1..11: note = Designed peptide K9
  SITE 4: note = Aib
  SITE 8: note = Aib
  SITE 9: note = Lys(HCl)
  SITE 11: note = Lol
XGLXGGLXXIX

SEQ ID NO: 6 - protein, 11 aa, synthetic construct
  SITE 1: note = 1 ottanoile Aib
  REGION 1..11: note = Designed peptide K9-NH2
  SITE 4: note = Aib
  SITE 8: note = Aib
  SITE 9: note = Lys(HCl)
XGLXGGLXXIL

SEQ ID NO: 7 - protein, 11 aa, synthetic construct
  SITE 1: note = 1 ottanoile Aib
  REGION 1..11: note = Designed peptide K256
  SITE 2: note = Lys(HCl)
  SITE 4: note = Aib
  SITE 5: note = Lys(HCl)
  SITE 6: note = Lys(HCl)
  SITE 8: note = Aib
  SITE 11: note = Lol
XXLXXXLXGIX

SEQ ID NO: 8 - protein, 11 aa, synthetic construct
  SITE 1: note = 1 ottanoile Aib
  REGION 1..11: note = Designed peptide K256-NH2
  SITE 2: note = Lys(HCl)
  SITE 4: note = Aib
  SITE 5: note = Lys(HCl)
  SITE 6: note = Lys(HCl)
  SITE 8: note = Aib
XXLXXXLXGIL

SEQ ID NO: 9-16 - skipped (8 entries)